European Patent Application EP 4 375 380 A1, published May 29, 2024. Title: 预防、缓解或治疗黏膜黏连的药物及其应用. Applicant: 上海循曜生物科技有限公司. The sequence listing filed with the application follows.

SEQUENCE LISTING (109 sequences)

SEQ ID NO: 1 - protein, 117 aa, synthetic construct
EVQLQQSGPELVKPGASMKISCKASGYSFTGYPMNWVRQSHVKNLEWIGVINPYNGGTSYNQKFKGKATLTVDKSSSTAYIELLSLTSDDSAVYYCARGGVRPFAYWGQGTLVTVSA

SEQ ID NO: 2 - protein, 117 aa, synthetic construct
EVQLQQSGPELVKPGASMKISCKASGYSFTGYPMNWVKQTHGKNLEWIGLINPYNGGTSYNQKFKGKATLTVDKSSSTAYMELLSLTSDESAVYYCARGGVRPFDFWGQGTLVTVSA

SEQ ID NO: 3 - protein, 117 aa, synthetic construct
EVQLQQSGPELVKPGASMKISCKASGYSFTGYPMNWVRQSHGKNLEWIGVINSYNGGASYNQKFKGKATLTVDKSSNIVHMELLSLTSEDSAVYYCARGGVRPFAYWGQGTLVTVSA

SEQ ID NO: 4 - protein, 118 aa, synthetic construct
EVQLQQSGPELVKPGASMKISCKASGYSFTGYTMNWVKQSHGENLEWIGVINPYNGGTSYNQKFKGKATLTVDKSFSTAYMEILSLTSEDSAVYYCSRGGGNSWFAYWGQGTLVTVSA

SEQ ID NO: 5 - protein, 118 aa, synthetic construct
EVQLQQSGPELVKPGASMKISCKASGYAFTGYTMNWVKQSHGKNLDWIGVINGYNGGTSYNQKFKGKATLTVDKSSSTAYMELLSLTSEDSAIYYCARGGPTTGFVYWGQGTLVTVSA

SEQ ID NO: 6 - protein, 115 aa, synthetic construct
EVQLQQSGPELVKPGASVKISCKASGYTFTDYYMNWVKQSHGESLEWIGDINPNNGGATYNQKFEGKATLTVDKSSSTAYMELRSLTSEDSAVYYCGQLLGFASWGQGTLVTVSA

SEQ ID NO: 7 - protein, 117 aa, synthetic construct
QVQLVQSGAEVKKPGASVKVSCKASGYTFTGYPMNWVRQAPGQNLEWMGVINPYNGGTSYNQKFKGRVTLTRDKSASTAYMELSSLRSEDTAVYYCARGGVRPFAYWGQGTLVTVSS

SEQ ID NO: 8 - protein, 117 aa, synthetic construct
QVQLVQSGAEVKKPGASVKVSCKASGYTFTGYPMNWVRQAPGKRLEWMGVINPYNGGTSYNQKFKGRATLTVDTSASTAYMELSSLRSEDTAVYYCARGGVRPFAYWGQGTLVTVSS

SEQ ID NO: 9 - protein, 117 aa, synthetic construct
QVQLVQSGAEVKKPGASVKVSCKASGYTFTGYPMNWVRQAPGQNLEWMGVINPYNGGTSYNQKFKGRVTLTVDKSASTAYMELSSLRSEDTAVYYCARGGVRPFAYWGQGTLVTVSS

SEQ ID NO: 10 - protein, 117 aa, synthetic construct
QVQLVQSGAEVKKPGASVKVSCKASGYTFTGYPMNWVRQAPGKNLEWMGVINPYNGGTSYNQKFKGRATLTVDKSASTAYMELSSLRSEDTAVYYCARGGVRPFAYWGQGTLVTVSS

SEQ ID NO: 11 - protein, 117 aa, synthetic construct
QVQLVQSGAEVKKPGASVKVSCKASGYTFTGYPMNWVRQAPGKRLEWMGVINPYSGGTSYNQKFKGRATLTVDTSASTAYMELSSLRSEDTAVYYCARGGVRPFAYWGQGTLVTVSS

SEQ ID NO: 12 - protein, 117 aa, synthetic construct
QVQLVQSGAEVKKPGASVKVSCKASGYTFTGYPMNWVRQAPGKRLEWMGVINPYDGGTSYNQKFKGRATLTVDTSASTAYMELSSLRSEDTAVYYCARGGVRPFAYWGQGTLVTVSS

SEQ ID NO: 13 - protein, 117 aa, synthetic construct
QVQLVQSGAEVKKPGASVKVSCKASGYTFTGYPMNWVRQAPGKRLEWMGVINPYQGGTSYNQKFKGRATLTVDTSASTAYMELSSLRSEDTAVYYCARGGVRPFAYWGQGTLVTVSS

SEQ ID NO: 14 - protein, 117 aa, synthetic construct
QVQLVQSGAEVKKPGASVKVSCKASGYTFTGYPMNWVRQAPGKRLEWMGVINPYNAGTSYNQKFKGRATLTVDTSASTAYMELSSLRSEDTAVYYCARGGVRPFAYWGQGTLVTVSS

SEQ ID NO: 15 - protein, 117 aa, synthetic construct
QVQLVQSGAEVKKPGASVKVSCKASGYTFTGYPMNWVRQAPGKRLEWMGVINPYNVGTSYNQKFKGRATLTVDTSASTAYMELSSLRSEDTAVYYCARGGVRPFAYWGQGTLVTVSS

SEQ ID NO: 16 - protein, 106 aa, synthetic construct
DIQMTQTSSSFSVSLGDRVTITCKASEDIYNRLAWYQQKPGNAPRLLISGATSLETGVPSRFSGSGSGNDYTLSITSLQTEDVATYYCQQYWSTPTFGAGTKLELQ

SEQ ID NO: 17 - protein, 107 aa, synthetic construct
DIVMTQSQKFMSTSVGDRVSVTCKASQNVDTNVAWYQQKPGQSPKALIYSASYRYSGVPDRFTGSGSGTDFTLTISNVQSEDLAEYFCQQYDSYPYTFGGGTKLEIR

SEQ ID NO: 18 - protein, 106 aa, synthetic construct
DIVITQSPAIMSASPGEKVTMTCSARSSVSYMYWYQQKPGSSPRLLIYDTSKLASGVPVRFSGSGSGTSYSLTISRMEAEDAATYFCQQWSSYPPTFGGGTKLEIK

SEQ ID NO: 19 - protein, 106 aa, synthetic construct
DIQMTQTSSYLSVSLGGRVTITCKASDHINNWLAWYQQKPGNAPRLLISGATSLETGVPSRFSGSGSGTDYSLTITSLQTEDVATYYCQQYWSIPTFGGGTRLEIK

SEQ ID NO: 20 - protein, 106 aa, synthetic construct
DIQMTQTSSSFSVSLGDRVTITCKASEDIYNRLAWYQQKPGNAPRLLISGATSLETGVPSRFSGSGSGKDYTLSITSLQTEDVATYYCQQYWSTPTFGAGTKLELK

SEQ ID NO: 21 - protein, 112 aa, synthetic construct
DVVLTQTPLSLPVNIGDQASISCRSTQSLLNSDRFTYLDWYLQRPGQSPQLLIYLVSYRFSGVPDRFSGSGSGTDFTLKISRVEAEDLGLYYCLQSSYLPYTFGGGTKLEIK

SEQ ID NO: 22 - protein, 106 aa, synthetic construct
DIQMTQSPSSLSASVGDRVTITCKASEDIYNRLAWYQQKPGKAPKLLISGATSLETGVPSRFSGSGSGNDFTLTISSLQPEDFATYYCQQYWSTPTFGQGTKLEIK

SEQ ID NO: 23 - protein, 106 aa, synthetic construct
DIQMTQSPSSLSASVGDRVTITCKASEDIYNRLAWYQQKPGNAPKLLISGATSLETGVPSRFSGSGSGNDFTLTISSLQPEDFATYYCQQYWSTPTFGQGTKLEIK

SEQ ID NO: 24 - protein, 106 aa, synthetic construct
DIQMTQSPSSLSASVGDRVTITCKASEDIYNRLAWYQQKPGKAPKLLISGATSLETGVPSRFSGSGSGNDYTLTISSLQPEDFATYYCQQYWSTPTFGQGTKLEIK

SEQ ID NO: 25 - protein, 106 aa, synthetic construct
DIQMTQSPSSLSASVGDRVTITCKASEDIYNRLAWYQQKPGNAPKLLISGATSLETGVPSRFSGSGSGNDYTLTISSLQPEDFATYYCQQYWSTPTFGQGTKLEIK

SEQ ID NO: 26 - protein, 8 aa, synthetic construct
GYSFTGYP

SEQ ID NO: 27 - protein, 8 aa, synthetic construct
INPYNGGT

SEQ ID NO: 28 - protein, 10 aa, synthetic construct
ARGGVRPFAY

SEQ ID NO: 29 - protein, 10 aa, synthetic construct
ARGGVRPFDF

SEQ ID NO: 30 - protein, 8 aa, synthetic construct
INSYNGGA

SEQ ID NO: 31 - protein, 8 aa, synthetic construct
GYSFTGYT

SEQ ID NO: 32 - protein, 11 aa, synthetic construct
SRGGGNSWFAY

SEQ ID NO: 33 - protein, 8 aa, synthetic construct
GYAFTGYT

SEQ ID NO: 34 - protein, 8 aa, synthetic construct
INGYNGGT

SEQ ID NO: 35 - protein, 11 aa, synthetic construct
ARGGPTTGFVY

SEQ ID NO: 36 - protein, 8 aa, synthetic construct
GYTFTDYY

SEQ ID NO: 37 - protein, 8 aa, synthetic construct
INPNNGGA

SEQ ID NO: 38 - protein, 8 aa, synthetic construct
GQLLGFAS

SEQ ID NO: 39 - protein, 8 aa, synthetic construct
GYTFTGYP

SEQ ID NO: 40 - protein, 8 aa, synthetic construct
INPYSGGT

SEQ ID NO: 41 - protein, 8 aa, synthetic construct
INPYDGGT

SEQ ID NO: 42 - protein, 8 aa, synthetic construct
INPYQGGT

SEQ ID NO: 43 - protein, 8 aa, synthetic construct
INPYNAGT

SEQ ID NO: 44 - protein, 8 aa, synthetic construct
INPYNVGT

SEQ ID NO: 45 - protein, 6 aa, synthetic construct
EDIYNR

SEQ ID NO: 46 - protein, 8 aa, synthetic construct
QQYWSTPT

SEQ ID NO: 47 - protein, 6 aa, synthetic construct
QNVDTN

SEQ ID NO: 48 - protein, 9 aa, synthetic construct
QQYDSYPYT

SEQ ID NO: 49 - protein, 5 aa, synthetic construct
SSVSY

SEQ ID NO: 50 - protein, 9 aa, synthetic construct
QQWSSYPPT

SEQ ID NO: 51 - protein, 6 aa, synthetic construct
DHINNW

SEQ ID NO: 52 - protein, 8 aa, synthetic construct
QQYWSIPT

SEQ ID NO: 53 - protein, 11 aa, synthetic construct
QSLLNSDRFTY

SEQ ID NO: 54 - protein, 9 aa, synthetic construct
LQSSYLPYT

SEQ ID NO: 55 - protein, 25 aa, synthetic construct
EVQLQQSGPELVKPGASMKISCKAS

SEQ ID NO: 56 - protein, 25 aa, synthetic construct
EVQLQQSGPELVKPGASVKISCKAS

SEQ ID NO: 57 - protein, 25 aa, synthetic construct [sequence omitted]

SEQ ID NO: 58 - protein, 17 aa, synthetic construct
MNWVKQSHGENLEWIGV

SEQ ID NO: 59 - protein, 17 aa, synthetic construct
MNWVKQSHGESLEWIGD

SEQ ID NO: 60 - protein, 17 aa, synthetic construct
MNWVKQSHGKNLDWIGV

SEQ ID NO: 61 - protein, 17 aa, synthetic construct
MNWVKQTHGKNLEWIGL

SEQ ID NO: 62 - protein, 17 aa, synthetic construct
MNWVRQAPGKNLEWMGV

SEQ ID NO: 63 - protein, 17 aa, synthetic construct
MNWVRQAPGKRLEWMGV

SEQ ID NO: 64 - protein, 17 aa, synthetic construct
MNWVRQAPGQNLEWMGV

SEQ ID NO: 65 - protein, 17 aa, synthetic construct
MNWVRQSHGKNLEWIGV

SEQ ID NO: 66 - protein, 17 aa, synthetic construct
MNWVRQSHVKNLEWIGV

SEQ ID NO: 67 - protein, 38 aa, synthetic construct
SYNQKFKGRVTLTVDKSASTAYMELSSLRSEDTAVYYC

SEQ ID NO: 68 - protein, 38 aa, synthetic construct
SYNQKFKGKATLTVDKSFSTAYMEILSLTSEDSAVYYC

SEQ ID NO: 69 - protein, 38 aa, synthetic construct
SYNQKFKGKATLTVDKSSNIVHMELLSLTSEDSAVYYC

SEQ ID NO: 70 - protein, 38 aa, synthetic construct
SYNQKFKGKATLTVDKSSSTAYIELLSLTSDDSAVYYC

SEQ ID NO: 71 - protein, 38 aa, synthetic construct
SYNQKFKGKATLTVDKSSSTAYMELLSLTSDESAVYYC

SEQ ID NO: 72 - protein, 38 aa, synthetic construct
SYNQKFKGKATLTVDKSSSTAYMELLSLTSEDSAIYYC

SEQ ID NO: 73 - protein, 38 aa, synthetic construct
SYNQKFKGRATLTVDKSASTAYMELSSLRSEDTAVYYC

SEQ ID NO: 74 - protein, 38 aa, synthetic construct
SYNQKFKGRATLTVDTSASTAYMELSSLRSEDTAVYYC

SEQ ID NO: 75 - protein, 38 aa, synthetic construct
SYNQKFKGRVTLTRDKSASTAYMELSSLRSEDTAVYYC

SEQ ID NO: 76 - protein, 38 aa, synthetic construct
TYNQKFEGKATLTVDKSSSTAYMELRSLTSEDSAVYYC

SEQ ID NO: 77 - protein, 11 aa, synthetic construct
WGQGTLVTVSA

SEQ ID NO: 78 - protein, 11 aa, synthetic construct
WGQGTLVTVSS

SEQ ID NO: 79 - protein, 26 aa, synthetic construct [sequence omitted]

SEQ ID NO: 80 - protein, 26 aa, synthetic construct
DIQMTQTSSSFSVSLGDRVTITCKAS

SEQ ID NO: 81 - protein, 26 aa, synthetic construct
DIQMTQTSSYLSVSLGGRVTITCKAS

SEQ ID NO: 82 - protein, 26 aa, synthetic construct
DIVITQSPAIMSASPGEKVTMTCSAR

SEQ ID NO: 83 - protein, 26 aa, synthetic construct
DIVMTQSQKFMSTSVGDRVSVTCKAS

SEQ ID NO: 84 - protein, 26 aa, synthetic construct
DVVLTQTPLSLPVNIGDQASISCRST

SEQ ID NO: 85 - protein, 17 aa, synthetic construct
LAWYQQKPGKAPKLLIS

SEQ ID NO: 86 - protein, 17 aa, synthetic construct
LAWYQQKPGNAPKLLIS

SEQ ID NO: 87 - protein, 17 aa, synthetic construct
LAWYQQKPGNAPRLLIS

SEQ ID NO: 88 - protein, 17 aa, synthetic construct
LDWYLQRPGQSPQLLIY

SEQ ID NO: 89 - protein, 17 aa, synthetic construct
MYWYQQKPGSSPRLLIY

SEQ ID NO: 90 - protein, 17 aa, synthetic construct
VAWYQQKPGQSPKALIY

SEQ ID NO: 91 - protein, 36 aa, synthetic construct
KLASGVPVRFSGSGSGTSYSLTISRMEAEDAATYFC

SEQ ID NO: 92 - protein, 36 aa, synthetic construct
SLETGVPSRFSGSGSGKDYTLSITSLQTEDVATYYC

SEQ ID NO: 93 - protein, 36 aa, synthetic construct
SLETGVPSRFSGSGSGNDFTLTISSLQPEDFATYYC

SEQ ID NO: 94 - protein, 36 aa, synthetic construct
SLETGVPSRFSGSGSGNDYTLSITSLQTEDVATYYC

SEQ ID NO: 95 - protein, 36 aa, synthetic construct
SLETGVPSRFSGSGSGNDYTLTISSLQPEDFATYYC

SEQ ID NO: 96 - protein, 36 aa, synthetic construct
SLETGVPSRFSGSGSGTDYSLTITSLQTEDVATYYC

SEQ ID NO: 97 - protein, 36 aa, synthetic construct
YRFSGVPDRFSGSGSGTDFTLKISRVEAEDLGLYYC

SEQ ID NO: 98 - protein, 36 aa, synthetic construct
YRYSGVPDRFTGSGSGTDFTLTISNVQSEDLAEYFC

SEQ ID NO: 99 - protein, 10 aa, synthetic construct
FGAGTKLELK

SEQ ID NO: 100 - protein, 10 aa, synthetic construct
FGGGTKLEIK

SEQ ID NO: 101 - protein, 10 aa, synthetic construct
FGGGTKLEIR

SEQ ID NO: 102 - protein, 10 aa, synthetic construct
FGGGTRLEIK

SEQ ID NO: 103 - protein, 10 aa, synthetic construct
FGQGTKLEIK

SEQ ID NO: 104 - DNA, 22 bp, synthetic construct
  source 1..22: mol_type = other DNA
caggcattggtgccagtgaaca

SEQ ID NO: 105 - DNA, 22 bp, synthetic construct
  source 1..22: mol_type = other DNA
tggacctccatcctcacagtca

SEQ ID NO: 106 - DNA, 22 bp, synthetic construct
  source 1..22: mol_type = other DNA
tgctgacagaggcaccactgaa

SEQ ID NO: 107 - DNA, 23 bp, synthetic construct
  source 1..23: mol_type = other DNA
cagttgtacgtccagaggcatag

SEQ ID NO: 108 - DNA, 20 bp, synthetic construct
  source 1..20: mol_type = other DNA
ttgactcaacacgggaaacc

SEQ ID NO: 109 - DNA, 20 bp, synthetic construct
  source 1..20: mol_type = other DNA
agacaaatcgctccaccaac